European Patent Specification EP 3 307 782 B1, published February 26, 2025. Title: METHODS AND ANTIBODIES FOR MODULATION OF IMMUNORESPONSE. Applicant: Lu, Yen-Ta. The sequence listing filed with the application follows.

SEQUENCE LISTING (32 sequences)

SEQ ID NO: 1 - protein, 5 aa, Artificial
  H-CDR1
NYWIN

SEQ ID NO: 2 - protein, 10 aa, artificial
  H-CDR1
GFSLTSNSIS

SEQ ID NO: 3 - protein, 17 aa, artificial
  H-CDR2
NIYPSDTYINHNQKFKD

SEQ ID NO: 4 - protein, 16 aa, artificial
  H-CDR2
AIWSGGGTDYNSDLKS

SEQ ID NO: 5 - protein, 9 aa, artificial
  H-CDR3
SAYANYFDY

SEQ ID NO: 6 - protein, 10 aa, artificial
  H-CDR3
RGGYPYYFDY

SEQ ID NO: 7 - protein, 11 aa, artificial
  L-CDR1
RASQNIGTSIH

SEQ ID NO: 8 - protein, 17 aa, artificial
  L-CDR1
KSSQSLLYSENQENYLA

SEQ ID NO: 9 - protein, 7 aa, artificial
  L-CDR2
YASESIS

SEQ ID NO: 10 - protein, 7 aa, artificial
  L-CDR2
WASTRQS

SEQ ID NO: 11 - protein, 10 aa, artificial
  L-CDR3
QQSDSWPTLT

SEQ ID NO: 12 - protein, 9 aa, artificial
  L-CDR3
QQYYDTPLT

SEQ ID NO: 13 - protein, 118 aa, artificial
  Heavy chain variable region of the humanized anti-CD11b antibodies-VH1
QVQLVQSGAEVKKPGASVKVSCKASGYTFTNYWINWVRQAPGQGLEWMGNIYPSDTYINHNQKFKDRVTMTRDTSTSTVYMELSSLRSEDTAVYYCARSAYANYFDYWGQGTLVTVSS

SEQ ID NO: 14 - protein, 118 aa, artificial
  Heavy chain variable region of the humanized anti-CD11b antibodies-VH2
QVQLVQSGAEVKKPGSSVKVSCKASGGTFSNYWINWVRQAPGQGLEWMGNIYPSDTYINHNQKFKDRVTITADKSTSTAYMELSSLRSEDTAVYYCATSAYANYFDYWGQGTLVTVSS

SEQ ID NO: 15 - protein, 118 aa, artificial
  Heavy chain variable region of the humanized anti-CD11b antibodies-VH3
QVQLVQSGAEVKKPGASVKVSCKASGYTFTNYWINWVRQATGQGLEWMGNIYPSDTYINHNQKFKDRVTMTRNTSISTAYMELSSLRSEDTAVYYCARSAYANYFDYWGQGTLVTVSS

SEQ ID NO: 16 - protein, 118 aa, artificial
  Heavy chain variable region of the humanized anti-CD11b antibodies-VH4
QVQLVQSGAEVKKPGASVKVSCKASGYTFTNYWINWVRQAPGQRLEWMGNIYPSDTYINHNQKFKDRVTITRDTSASTAYMELSSLRSEDTAVYYCARSAYANYFDYWGQGTLVTVSS

SEQ ID NO: 17 - protein, 118 aa, artificial
  Heavy chain variable region of the humanized anti-CD11b antibodies-VH5
QVQLVQSGAEVKKPGATVKISCKVSGYTFTNYWINWVQQAPGKGLEWMGNIYPSDTYINHNQKFKDRVTITADTSTDTAYMELSSLRSEDTAVYYCARSAYANYFDYWGQGTLVTVSR

SEQ ID NO: 18 - protein, 117 aa, artificial
  Heavy chain variable region of the humanized anti-CD11b antibodies-HC1
QVQLQESGPGLVKPSETLSLTCTVSGFSLTSNSISWIRQPPGKGLEWIGAIWSGGGTDYNSDLKSRVTISVDTSKNQFSLKLSSVTAADTAVYYCARGGYPYYFDYWGQGTLVTVSS

SEQ ID NO: 19 - protein, 117 aa, artificial
  Heavy chain variable region of the humanized anti-CD11b antibodies-HC2
QVQLQESGPGLVKPSGTLSLTCAVYGFSLTSNSISWIRQPPGKGLEWIGAIWSGGGTDYNSDLKSRVTISVDTSKNQFSLKLSSVTAADTAVYYCARGGYPYYFDYWGQGTMVTVSS

SEQ ID NO: 20 - protein, 117 aa, artificial
  Heavy chain variable region of the humanized anti-CD11b antibodies-HC3
QVQLQQWGAGLLKPSETLSLTCAVYGFSLTSNSISWIRQPPGKGLEWIGAIWSGGGTDYNSDLKSRVTISVDTSKNQFSLKLSSVTAADTAVYYCARGGYPYYFDYWGQGTLVTVSS

SEQ ID NO: 21 - protein, 117 aa, artificial
  Heavy chain variable region of the humanized anti-CD11b antibodies-HC4
EVQLVESGGGLVQPGGSLRLSCAASGFSLTSNSISWVRQAPGKGLEWVSAIWSGGGTDYNSDLKSRFTISRDNSKNTLYLQMNSLRAEDTAVYYCARGGYPYYFDYWGQGTLVTVSS

SEQ ID NO: 22 - protein, 117 aa, artificial
  Heavy chain variable region of the humanized anti-CD11b antibodies-HC5
EVQLVETGGGLIQPGGSLRLSCAASGFSLTSNSISWVRQAPGKGLEWVSAIWSGGGTDYNSDLKSRFTISRDNSKNTLYLQMNSLRAEDTAVYYCARGGYPYYFDYWGQGTLVTVSS

SEQ ID NO: 23 - protein, 108 aa, artificial
  Light chain variable region of the humanized anti-CD11b antibodies-VL1
EIVLTQSPDFQSVTPKEKVTITCRASQNIGTSIHWYQQKPDQSPKLLIKYASESISGVPSRFSGSGSGTDFTLTINSLEAEDAATYYCQQSDSWPTLTFGQGTKVEIK

SEQ ID NO: 24 - protein, 108 aa, artificial
  Light chain variable region of the humanized anti-CD11b antibodies-VL2
EIVMTQSPATLSVSPGERATLSCRASQNIGTSIHWYQQKPGQAPRLLIYYASESISGIPARFSGSGSGTEFTLTISSLQSEDFAVYYCQQSDSWPTLTFGQGTKLEIK

SEQ ID NO: 25 - protein, 108 aa, artificial
  Light chain variable region of the humanized anti-CD11b antibodies-VL3
DIQMTQSPSSLSASVGDRVTITCRASQNIGTSIHWYQQKPGKAPKLLIYYASESISGVPSRFSGSGSGTDFTLTISSLQPEDFATYYCQQSDSWPTLTFGGGTKVEIK

SEQ ID NO: 26 - protein, 108 aa, artificial
  Light chain variable region of the humanized anti-CD11b antibodies-VL4
EIVLTQSPATLSLSPGERATLSCRASQNIGTSIHWYQQKPGQAPRLLIYYASESISGIPARFSGSGSGTDFTLTISSLEPEDFAVYYCQQSDSWPTLTFGGGTKVEIK

SEQ ID NO: 27 - protein, 108 aa, artificial
  Light chain variable region of the humanized anti-CD11b antibodies-VL5
EIVLTQSPGTLSLSPGERATLSCRASQNIGTSIHWYQQKPGQAPRLLIYYASESISGIPDRFSGSGSGTDFTLTISRLEPEDFAVYYCQQSDSWPTLTFGQGTKLEIK

SEQ ID NO: 28 - protein, 113 aa, artificial
  Light chain variable region of the humanized anti-CD11b antibodies-LC1
DIVMTQSPDSLAVSLGERATINCKSSQSLLYSENQENYLAWYQQKPGQPPKLLIYWASTRQSGVPDRFSGSGSGTDFTLTISSLQAEDVAVYYCQQYYDTPLTFGQGTKVEIK

SEQ ID NO: 29 - protein, 113 aa, artificial
  Light chain variable region of the humanized anti-CD11b antibodies-LC2
DIVMTQSPLSLPVTPGEPASISCKSSQSLLYSENQENYLAWYLQKPGQSPQLLIYWASTRQSGVPDRFSGSGSGTDFTLKISRVEAEDVGVYYCQQYYDTPLTFGGGTKVEIK

SEQ ID NO: 30 - protein, 113 aa, artificial
  Light chain variable region of the humanized anti-CD11b antibodies-LC3
DIVMTQSPLSLSVTPGQPASISCKSSQSLLYSENQENYLAWYLQKPGQSPQLLIYWASTRQSGVPDRFSGSGSGTDFTLKISRVEAEDVGVYYCQQYYDTPLTFGQGTKVEIK

SEQ ID NO: 31 - protein, 113 aa, artificial
  Light chain variable region of the humanized anti-CD11b antibodies-LC4
DVVMTQSPLSLPVTLGQPASISCKSSQSLLYSENQENYLAWFQQRPGQSPRRLIYWASTRQSGVPDRFSGSGSGTDFTLKISRVEAEDVGVYYCQQYYDTPLTFGQGTKLEIK

SEQ ID NO: 32 - protein, 113 aa, artificial
  Light chain variable region of the humanized anti-CD11b antibodies-LC5
DIVMTQTPLSSPVTLGQPASISCKSSQSLLYSENQENYLAWLQQRPGQPPRLLIYWASTRQSGVPDRFSGSGAGTDFTLKISRVEAEDVGVYYCQQYYDTPLTFGQGTKLEIK